European Patent Application EP 4 545 547 A1, published April 30, 2025. Title: INSECT NEUROPEPTIDES 4. Applicant: SOLASTA Bio Limited. The sequence listing filed with the application follows.

SEQUENCE LISTING (16 sequences)

SEQ ID NO: 1 - protein, 10 aa, synthetic construct
  source 1..10: note = Z peptide
GGSMTFSPRL

SEQ ID NO: 2 - protein, 10 aa, synthetic construct
  source 1..10: note = SB-P-81
  MOD_RES 10: note = leucinamide
GGSMTFSPRL

SEQ ID NO: 3 - protein, 11 aa, synthetic construct
  source 1..11: note = SB-P-47
  MOD_RES 11: note = leucinamide
  MOD_RES 1: note = pyroglutamyl-alanine
AIMARPQVPRL

SEQ ID NO: 4 - protein, 8 aa, synthetic construct
  source 1..8: note = SB-P-49
  MOD_RES 8: note = leucinamide
SVPFKPRL

SEQ ID NO: 5 - protein, 19 aa, synthetic construct
  source 1..19: note = SB-P-51
  MOD_RES 19: note = leucinamide
LRQLQSNGEPAYRVRTPRL

SEQ ID NO: 6 - protein, 16 aa, synthetic construct
  source 1..16: note = SB-P-80
  MOD_RES 16: note = leucinamide
NADEDQQQSVDFTPRL

SEQ ID NO: 7 - protein, 12 aa, synthetic construct
  source 1..12: note = SB-P-46
  MOD_RES 12: note = leucinamide
SPPYSPPFSPRL

SEQ ID NO: 8 - protein, 8 aa, synthetic construct
  source 1..8: note = SB-P-70
  MOD_RES 8: note = glycinamide
KVKFSAWG

SEQ ID NO: 9 - protein, 10 aa, synthetic construct
  source 1..10: note = SB-P-65
  MOD_RES 10: note = glycinamide
RQKTVFSSWG

SEQ ID NO: 10 - protein, 7 aa, synthetic construct
  source 1..7: note = SB-P-66
  MOD_RES 7: note = glycinamide
PAFSSWG

SEQ ID NO: 11 - protein, 9 aa, synthetic construct
  source 1..9: note = SB-P-86
  MOD_RES 9: note = glycinamide
  MOD_RES 1: note = pyroglutamyl-leucine
LTFTSSWGG

SEQ ID NO: 12 - protein, 8 aa, synthetic construct
  source 1..8: note = SB-P-039
  MOD_RES 1: note = palmitoyl-glutamine
  MOD_RES 8: note = tryptophanamide
QLTFSPDW

SEQ ID NO: 13 - protein, 7 aa, synthetic construct
  source 1..7: note = SB-P-042
  MOD_RES 1: note = pyroglutamyl-leucine
  MOD_RES 7: note = tryptophanamide
LTFSPDW

SEQ ID NO: 14 - protein, 6 aa, synthetic construct
  source 1..6: note = SB-P-69
  MOD_RES 6: note = glycinamide
NFSPWG

SEQ ID NO: 15 - protein, 19 aa, synthetic construct
  source 1..19: note = SB-P-48
  MOD_RES 19: note = leucinamide
EQNVQSNGEPAYRVRTPRL

SEQ ID NO: 16 - protein, 8 aa, synthetic construct
  source 1..8: note = SB-P-41
  MOD_RES 8: note = tryptophanamide
QLTFSPDW